European Patent Specification EP 4 185 700 B1, published December 17, 2025. Title: Optimized SLC13A5 Genes and Expression Cassettes and Their Use. Applicant: The University of North Carolina at Chapel Hill Bailey, Rachel Gray, Steven J. The sequence listing filed with the application follows.

SEQUENCE LISTING (5 sequences)

SEQ ID NO: 1 - DNA, 1704 bp, Homo sapiens
atggcctcggcgctgagctatgtctccaagttcaagtccttcgtgatcttgttcgtcaccccgctcctgctgctgccactcgtcattctgatgcccgccaagtttgtcaggtgtgcctacgtcatcatcctcatggccatttactggtgcacagaagtcatccctctggctgtcacctctctcatgcctgtcttgcttttcccactcttccagattctggactccaggcaggtgtgtgtccagtacatgaaggacaccaacatgctgttcctgggcggcctcatcgtggccgtggctgtggagcgctggaacctgcacaagaggatcgccctgcgcacgctcctctgggtgggggccaagcctgcacggctgatgctgggcttcatgggcgtcacagccctcctgtccatgtggatcagtaacacggcaaccacggccatgatggtgcccatcgtggaggccatattgcagcagatggaagccacaagcgcagccaccgaggccggcctggagctggtggacaagggcaaggccaaggagctgccagggagtcaagtgatttttgaaggccccactctggggcagcaggaagaccaagagcggaagaggttgtgtaaggccatgaccctgtgcatctgctacgcggccagcatcgggggcaccgccaccctgaccgggacgggacccaacgtggtgctcctgggccagatgaacgagttgtttcctgacagcaaggacctcgtgaactttgcttcctggtttgcatttgcctttcccaacatgctggtgatgctgctgttcgcctggctgtggctccagtttgtttacatgagattcaattttaaaaagtcctggggctgcgggctagagagcaagaaaaacgagaaggctgccctcaaggtgctgcaggaggagtaccggaagctggggcccttgtccttcgcggagatcaacgtgctgatctgcttcttcctgctggtcatcctgtggttctcccgagaccccggcttcatgcccggctggctgactgttgcctgggtggagggtgagacaaagtatgtctccgatgccactgtggccatctttgtggccaccctgctattcattgtgccttcacagaagcccaagtttaacttccgcagccagactgaggaagaaaggaaaactccattttatccccctcccctgctggattggaaggtaacccaggagaaagtgccctggggcatcgtgctgctactagggggcggatttgctctggctaaaggatccgaggcctcggggctgtccgtgtggatggggaagcagatggagcccttgcacgcagtgcccccggcagccatcaccttgatcttgtccttgctcgttgccgtgttcactgagtgcacaagcaacgtggccaccaccaccttgttcctgcccatctttgcctccatgtctcgctccatcggcctcaatccgctgtacatcatgctgccctgtaccctgagtgcctcctttgccttcatgttgcctgtggccacccctccaaatgccatcgtgttcacctatgggcacctcaaggttgctgacatggtgaaaacaggagtcataatgaacataattggagtcttctgtgtgtttttggctgtcaacacctggggacgggccatatttgacttggatcatttccctgactgggctaatgtgacacatattgagact

SEQ ID NO: 2 - DNA, 1704 bp, Artificial Sequence
  Human codon-optimized SLC13A5 open reading frame
atggcctcggcgttgagctacgtgtccaagttcaagtcctttgtgatcctgtttgtgacccctctcttgctcctgccactcgtgattctgatgccggccaagtttgtgcgctgcgcctacgtgatcatcctgatggcaatctactggtgtaccgaagtcatccccctcgccgtgacttctcttatgccggtgctgctgttcccgctgttccaaatcctcgacagccgccaggtctgcgtgcagtacatgaaggacaccaacatgctgttcctgggcggcctgattgtggccgtggcagtggagcggtggaacctccacaagcgcatcgccctgaggactctgctctgggtcggcgctaagccagcgcggctgatgctggggttcatgggagtgaccgcgctgctctccatgtggatcagcaacaccgccactaccgccatgatggtcccgatcgtggaagccattctgcaacagatggaagctacttccgccgccactgaagcgggactggaactggtggacaagggaaaggccaaggaactgcccggttcacaagtcatcttcgagggaccaactctgggccagcaggaggaccaagagcgcaagcggctgtgcaaggccatgaccttgtgtatctgctacgccgcttcgatcggaggcactgccaccctgaccgggactggacccaacgtcgtgctgctgggacagatgaacgagctgttcccggattccaaggaccttgtgaacttcgcgtcgtggttcgccttcgcattccctaacatgctcgtgatgctgctctttgcatggctgtggctgcagttcgtgtatatgcggtttaacttcaagaagtcctggggatgcggtctggaatccaagaagaacgagaaggccgcgcttaaggtcctccaggaagaataccggaaattggggccgctgagcttcgccgagatcaacgtgctcatctgtttcttcctgctggtcatcctgtggttctcaagagatcctggtttcatgccggggtggctcactgtggcctgggtcgaaggagaaaccaaatacgtgtcggatgcgactgtggcaatctttgtcgccacgctcctgttcatcgtgccttcccaaaagcctaagttcaacttccgctcccaaaccgaagaggagcgcaaaacaccgttttaccctccacctctgttggactggaaagtcacccaggaaaaggtcccatggggcatcgtgctcctgctgggcggaggtttcgccctggctaagggcagcgaagccagcggtctgtccgtgtggatgggaaaacagatggagccgctgcacgctgtgccccctgctgccatcactctcattctgtccctgcttgtcgccgtgtttaccgagtgcacctccaacgtcgctaccactactctgttcttgcccatcttcgcctcgatgtcgagatccatcggcctgaaccccctctacattatgctgccgtgcaccttgtccgcctccttcgcgttcatgctgcctgtggcgactcccccgaatgctattgtgttcacctacggccatctcaaggtcgcagacatggtcaagaccggagtgatcatgaacattattggcgtgttctgcgtgttcttggccgtgaatacctggggtagagcaattttcgaccttgaccacttcccggactgggccaacgtgacccatatcgaaact

SEQ ID NO: 3 - DNA, 326 bp, Artificial Sequence
  UsP promoter
gggcggagttagggcggagccaatcagcgtgcgccgttccgaaagttgccttttatggctgggcggagaatgggcggtgaacgccgatgattatataaggacgcgccgggtgtggcacagctagttccgtcgcagccgggatttgggtcgcggttcttgtttgtggatccctgtgatcgtcacttggtaagtcactgactgtctatgcctgggaaagggtgggcaggagatggggcagtgcaggaaaagtggcactatgaaccctgcagccctaggaatgcatctagacaattgtactaaccttcttctctttcctctcctgacag

SEQ ID NO: 4 - DNA, 48 bp, Artificial Sequence
  SpA
aataaagagctcagatgcatcgatcagagtgtgttggttttttgtgtg

SEQ ID NO: 5 - DNA, 2145 bp, Artificial Sequence
  Human SLC13A5 expression cassette excluding ITRs
ggttcggtaccgggcggagttagggcggagccaatcagcgtgcgccgttccgaaagttgccttttatggctgggcggagaatgggcggtgaacgccgatgattatataaggacgcgccgggtgtggcacagctagttccgtcgcagccgggatttgggtcgcggttcttgtttgtggatccctgtgatcgtcacttggtaagtcactgactgtctatgcctgggaaagggtgggcaggagatggggcagtgcaggaaaagtggcactatgaaccctgcagccctaggaatgcatctagacaattgtactaaccttcttctctttcctctcctgacagtccggaaccggtgccaccatggcctcggcgttgagctacgtgtccaagttcaagtcctttgtgatcctgtttgtgacccctctcttgctcctgccactcgtgattctgatgccggccaagtttgtgcgctgcgcctacgtgatcatcctgatggcaatctactggtgtaccgaagtcatccccctcgccgtgacttctcttatgccggtgctgctgttcccgctgttccaaatcctcgacagccgccaggtctgcgtgcagtacatgaaggacaccaacatgctgttcctgggcggcctgattgtggccgtggcagtggagcggtggaacctccacaagcgcatcgccctgaggactctgctctgggtcggcgctaagccagcgcggctgatgctggggttcatgggagtgaccgcgctgctctccatgtggatcagcaacaccgccactaccgccatgatggtcccgatcgtggaagccattctgcaacagatggaagctacttccgccgccactgaagcgggactggaactggtggacaagggaaaggccaaggaactgcccggttcacaagtcatcttcgagggaccaactctgggccagcaggaggaccaagagcgcaagcggctgtgcaaggccatgaccttgtgtatctgctacgccgcttcgatcggaggcactgccaccctgaccgggactggacccaacgtcgtgctgctgggacagatgaacgagctgttcccggattccaaggaccttgtgaacttcgcgtcgtggttcgccttcgcattccctaacatgctcgtgatgctgctctttgcatggctgtggctgcagttcgtgtatatgcggtttaacttcaagaagtcctggggatgcggtctggaatccaagaagaacgagaaggccgcgcttaaggtcctccaggaagaataccggaaattggggccgctgagcttcgccgagatcaacgtgctcatctgtttcttcctgctggtcatcctgtggttctcaagagatcctggtttcatgccggggtggctcactgtggcctgggtcgaaggagaaaccaaatacgtgtcggatgcgactgtggcaatctttgtcgccacgctcctgttcatcgtgccttcccaaaagcctaagttcaacttccgctcccaaaccgaagaggagcgcaaaacaccgttttaccctccacctctgttggactggaaagtcacccaggaaaaggtcccatggggcatcgtgctcctgctgggcggaggtttcgccctggctaagggcagcgaagccagcggtctgtccgtgtggatgggaaaacagatggagccgctgcacgctgtgccccctgctgccatcactctcattctgtccctgcttgtcgccgtgtttaccgagtgcacctccaacgtcgctaccactactctgttcttgcccatcttcgcctcgatgtcgagatccatcggcctgaaccccctctacattatgctgccgtgcaccttgtccgcctccttcgcgttcatgctgcctgtggcgactcccccgaatgctattgtgttcacctacggccatctcaaggtcgcagacatggtcaagaccggagtgatcatgaacattattggcgtgttctgcgtgttcttggccgtgaatacctggggtagagcaattttcgaccttgaccacttcccggactgggccaacgtgacccatatcgaaacttgataggcggccgcggagctctcgagaggcctaataaagagctcagatgcatcgatcagagtgtgttggttttttgtgtgacgcgt